European Patent Specification EP 3 986 374 B1, published January 28, 2026. Title: LIPID NANOCAPSULES CHARGED WITH INCRETIN MIMETICS. Applicant: UNIVERSITÉ CATHOLIQUE DE LOUVAIN BELOQUI Ana XU Yining PRÉAT Véronique CANI Patrice. The sequence listing filed with the application follows.

SEQUENCE LISTING (16 sequences)

SEQ ID NO: 1 - DNA, 23 bp, Artificial Sequence
  Rpl19f
gaaggtcaaagggaatgtgttca

SEQ ID NO: 2 - DNA, 21 bp, Artificial Sequence
  Rpl19r
ccttgtctgccttcagcttgt

SEQ ID NO: 3 - DNA, 20 bp, Artificial Sequence
  F4/80f
tgacaaccagacggcttgtg

SEQ ID NO: 4 - DNA, 22 bp, Artificial Sequence
  F4/80r
gcaggcgaggaaaagatagtgt

SEQ ID NO: 5 - DNA, 24 bp, Artificial Sequence
  Cd11cf
acgtcagtacaaggagatgttgga

SEQ ID NO: 6 - DNA, 26 bp, Artificial Sequence
  Cd11cr
atcctattgcagaatgcttctttacc

SEQ ID NO: 7 - DNA, 19 bp, Artificial Sequence
  Mcp1f
gcagttaacgccccactca

SEQ ID NO: 8 - DNA, 22 bp, Artificial Sequence
  Mcp1r
tccagcctactcattgggatca

SEQ ID NO: 9 - DNA, 21 bp, Artificial Sequence
  Tnfaf
tcgagtgacaagcctgtagcc

SEQ ID NO: 10 - DNA, 19 bp, Artificial Sequence
  Tnfar
ttgagatccatgccgttgg

SEQ ID NO: 11 - DNA, 20 bp, Artificial Sequence
  Fasnf
caggcccctctgttaattgg

SEQ ID NO: 12 - DNA, 20 bp, Artificial Sequence
  Fasnr
tccagggataacagcacctt

SEQ ID NO: 13 - DNA, 23 bp, Artificial Sequence
  Ppargf
ctgctcaagtatggtgtccatga

SEQ ID NO: 14 - DNA, 26 bp, Artificial Sequence
  Ppargr
tgagatgaggactccatctttattca

SEQ ID NO: 15 - DNA, 24 bp, Artificial Sequence
  Cpt1a
agaccgtgaggaactcaaacctat

SEQ ID NO: 16 - DNA, 18 bp, Artificial Sequence
  Cpt1ar
tgaagagtcgctcccact